European Patent Application EP 4 289 961 A1, published December 13, 2023. Title: METHOD FOR SYNTHESIZING (1R,2R)-AMPP BY USING ENZYME CASCADE REACTION. Applicant: ZHEJIANG APELOA KANGYU PHARMACEUTICAL CO., LTD. APELOA PHARMACEUTICAL CO., LTD. The sequence listing filed with the application follows.

SEQUENCE LISTING (8 sequences)

SEQ ID NO: 1 - protein, 663 aa, Artificial Sequence
  Amino acid sequence of Escherichia coli transketolase
MSSRKELANAIRALSMDAVQKAKSGHPGAPMGMADIAEVLWRDFLKHNPQNPSWADRDRFVLSNGHGSMLIYSLLHLTGYDLPMEELKNFRQLHSKTPGHPEVGYTAGVETTTGPLGQGIANAVGMAIAEKTLAAQFNRPGHDIVDHYTYAFMGDGCMMEGISHEVCSLAGTLKLGKLIAFYDDNGISIDGHVEGWFTDDTAMRFEAYGWHVIRDIDGHDAASIKRAVEEARAVTDKPSLLMCKTIIGFGSPNKAGTHDSHGAPLGDAEIALTREQLGWKYAPFEIPSEIYAQWDAKEAGQAKESAWNEKFAAYAKAYPQEAAEFTRRMKGEMPSDFDAKAKEFIAKLQANPAKIASRKASQNAIEAFGPLLPEFLGGSADLAPYNLTLWSGSKAINEDAAGNYIHYGVREFGMTAIANGISLHGGFLPYTSTFLMFVEYARNAVRMAALMKQRQVMVYTHDSIGLGETGPTHQPVEQVASLRVTPNMSTWRPCDQVESAVAWKYGVERQDGPTALILSQQNLAQQERTEEQLANIARGGYVLKDCAGQPELIFIATGSEVELAVAAYEKLTAEGVKARVVSMPSTDAFDKQDAAYRESVLPKAVTARVAVEAGIADYWYKYVGLNGAIVGMTTFGESAPAELLFEEFGFTVDNVVAKAKELL

SEQ ID NO: 2 - DNA, 1992 bp, Artificial Sequence
  Nucleotide sequence of E. coli transketolase
atgtcctcacgtaaagagcttgccaatgctattcgtgcgctgagcatggacgcagtacagaaagccaaatccggtcacccgggtgcccctatgggtatggctgacattgccgaagtcctgtggcgtgatttcctgaaacacaacccgcagaatccgtcctgggctgaccgtgaccgcttcgtgctgtccaacggccacggctccatgctgatctacagcctgctgcacctcaccggttacgatctgccgatggaagaactgaaaaacttccgtcagctgcactctaaaactccgggtcacccggaagtgggttacaccgctggtgtggaaaccaccaccggtccgctgggtcagggtattgccaacgcagtcggtatggcgattgcagaaaaaacgctggcggcgcagtttaaccgtccgggccacgacattgtcgaccactacacctacgccttcatgggcgacggctgcatgatggaaggcatctcccacgaagtttgctctctggcgggtacgctgaagctgggtaaactgattgcattctacgatgacaacggtatttctatcgatggtcacgttgaaggctggttcaccgacgacaccgcaatgcgtttcgaagcttacggctggcacgttattcgcgacatcgacggtcatgacgcggcatctatcaaacgcgcagtagaagaagcgcgcgcagtgactgacaaaccttccctgctgatgtgcaaaaccatcatcggtttcggttccccgaacaaagccggtacccacgactcccacggtgcgccgctgggcgacgctgaaattgccctgacccgcgaacaactgggctggaaatatgcgccgttcgaaatcccgtctgaaatctatgctcagtgggatgcgaaagaagcaggccaggcgaaagaatccgcatggaacgagaaattcgctgcttacgcgaaagcttatccgcaggaagccgctgaatttacccgccgtatgaaaggcgaaatgccgtctgacttcgacgctaaagcgaaagagttcatcgctaaactgcaggctaatccggcgaaaatcgccagccgtaaagcgtctcagaatgctatcgaagcgttcggtccgctgttgccggaattcctcggcggttctgctgacctggcgccgtataacctgaccctgtggtctggttctaaagcaatcaacgaagatgctgcgggtaactacatccactacggtgttcgcgagttcggtatgaccgcgattgctaacggtatctccctgcacggtggcttcctgccgtacacctccaccttcctgatgttcgtggaatacgcacgtaacgccgtacgtatggctgcgctgatgaaacagcgtcaggtgatggtttacacccacgactccatcggtctgggcgaaaccggcccgactcaccagccggttgagcaggtcgcttctctgcgcgtaaccccgaacatgtctacatggcgtccgtgtgaccaggttgaatccgcggtcgcgtggaaatacggtgttgagcgtcaggacggcccgaccgcactgatcctctcccaacagaacctggcgcagcaggaacgaactgaagagcaactggcaaacatcgcgcgcggtggttatgtgctgaaagactgcgccggtcagccggaactgattttcatcgctaccggttcagaagttgaactggctgttgctgcctacgaaaaactgactgccgaaggcgtgaaagcgcgcgtggtgtccatgccgtctaccgacgcatttgacaagcaggatgctgcttaccgtgaatccgtactgccgaaagcggttactgcacgcgttgctgtagaagcgggtattgctgactactggtacaagtatgttggcctgaacggtgctatcgtcggtatgaccaccttcggtgaatctgctccggcagagctgctgtttgaagagttcggcttcactgttgataacgttgttgcgaaagcaaaagaactgctgtaa

SEQ ID NO: 3 - protein, 330 aa, Artificial Sequence
  Amino acid sequence of the transaminase ATA117
MAFSADTSEIVYTHDTGLDYITYSDYELDPANPLAGGAAWIEGAFVPPSEARISIFDQGYLHSDVTYTVFHVWNGNAFRLDDHIERLFSNAESMRIIPPLTQDEVKEIALELVAKTELREAFVSVSITRGYSSTPGERDITKHRPQVYMYAVPYQWIVPFDRIRDGVHAMVAQSVRRTPRSSIDPQVKNFQWGDLIRAVQETHDRGFEAPLLLDGDGLLAEGSGFNVVVIKDGVVRSPGRAALPGITRKTVLEIAESLGHEAILADITLAELLDADEVLGCTTAGGVWPFVSVDGNPISDGVPGPVTQSIIRRYWELNVESSSLLTPVQY

SEQ ID NO: 4 - DNA, 990 bp, Artificial Sequence
  Nucleotide sequence of the transaminase ATA117
atggcatttagcgcggataccagcgaaatcgtctatacccacgataccggtctggattacatcacctacagcgattacgaactggatccggcaaatccgttagcaggcggcgcagcttggattgaaggcgcatttgttccgccgtctgaagcgcgtattagcatcttcgatcagggctatctgcatagcgacgttacctataccgtcttccacgtttggaacggtaacgcatttcgtctggacgatcacatcgaacgtctgttcagcaacgccgaaagtatgcgtattattccgccgctgacccaagacgaagtcaaagaaatcgcgctggaactggttgcaaaaaccgaactgcgcgaagcgtttgttagcgttagcattacccgcggttatagtagtaccccgggcgaacgcgatattaccaaacatcgtccgcaggtctacatgtacgctgttccgtaccagtggatcgttccgtttgatcgtattcgcgacggcgttcacgcaatggttgcacagagcgtgcgtcgtaccccgcgtagcagcatcgatccgcaggtcaaaaacttccagtggggcgatttaattcgcgcagttcaggaaacccacgatcgcggttttgaagcaccgttactgttagacggcgacggtttactggcagaaggtagcggctttaacgtcgtcgtcattaaagatggggttgttcgttctccgggtcgtgcagcattaccgggtattacccgcaaaaccgttctggaaattgcggaatccctgggtcatgaagcgattctggcggatattaccttagcggaactgctggacgcagacgaagttttaggttgtaccaccgctggcggcgtttggccgtttgttagcgttgacggcaatccgattagcgatggtgttccgggtccggttacccaaagcattattcgtcgctactgggagctgaacgttgaaagtagcagcctgttaaccccggttcagtat

SEQ ID NO: 5 - DNA, 1992 bp, Artificial Sequence
  Nucleotide sequence of the transketolase EcTK1_YYH
atgtcctcacgtaaagagcttgccaatgctattcgtgcgctgagcatggacgcagtacagaaagccaaatccggttatccgggtgcccctatgggtatggctgacattgccgaagtcctgtggcgtgatttcctgaaacacaacccgcagaatccgtcctgggctgaccgtgaccgcttcgtgctgtccaacggccacggctccatgctgatctacagcctgctgcacctcaccggttacgatctgccgatggaagaactgaaaaacttccgtcagctgcactctaaaactccgggtcacccggaagtgggttacaccgctggtgtggaaaccaccaccggtccgctgggtcagggtattgccaacgcagtcggtatggcgattgcagaaaaaacgctggcggcgcagtttaaccgtccgggccacgacattgtcgaccactacacctacgccttcatgggcgacggctgcatgatggaaggcatctcccacgaagtttgctctctggcgggtacgctgaagttgggtaaactgattgcattctacgatgacaacggtatttctatcgatggtcacgttgaaggctggttcaccgacgacaccgcaatgcgtttcgaagcttacggctggcacgttattcgcgacatcgacggtcatgacgcggcatctatcaaacgcgcagtagaagaagcgcgcgcagtgactgacaaaccttccctgctgatgtgcaaaaccatcatcggtttcggttccccgaacaaagccggtacccacgactcccacggtgcgccgctgggcgacgctgaaattgccctgacccgcgaacaactgggctggaaatatgcgccgttcgaaatcccgtctgaaatctatgctcagtgggatgcgaaagaagcaggccaggcgaaagaatccgcatggaacgagaaattcgctgcttacgcgaaagcttatccgcaggaagccgctgaatttacccgccgtatgaaaggcgaaatgccgtctgacttcgacgctaaagcgaaagagttcatcgctaaactgcaggctaatccggcgaaaatcgccagccgtaaagcgtctcagaatgctatcgaagcgttcggtccgctgttgccggaattcctcggcggttctgctgacctggcgccgtataacctgaccctgtggtctggttctaaagcaatcaacgaagatgctgcgggtaactacatccactacggtgttcgcgagttcggtatgaccgcgattgctaacggtatctccctgcacggtggcttcctgccgtacacctccacctatctgatgttcgtggaatacgcacgtaacgccgtacgtatggctgcgctgatgaaacagcgtcaggtgatggtttacacccacgactccatcggtcatggcgaaaccggcccgactcaccagccggttgagcaggtcgcttctctgcgcgtaaccccgaacatgtctacatggcgtccgtgtgaccaggttgaatccgcggtcgcgtggaaatacggtgttgagcgtcaggacggcccgaccgcactgatcctctcccaacagaacctggcgcagcaggaacgaactgaagagcaactggcaaacatcgcgcgcggtggttatgtgctgaaagactgcgccggtcagccggaactgattttcatcgctaccggttcagaagttgaactggctgttgctgcctacgaaaaactgactgccgaaggcgtgaaagcgcgcgtggtgtccatgccgtctaccgacgcatttgacaagcaggatgctgcttaccgtgaatccgtactgccgaaagcggttactgcacgcgttgctgtagaagcgggtattgctgactactggtacaagtatgttggcctgaacggtgctatcgtcggtatgaccaccttcggtgaatctgctccggcagagctgctgtttgaagagttcggcttcactgttgataacgttgttgcgaaagcaaaagaactgctgtaa

SEQ ID NO: 6 - DNA, 993 bp, Artificial Sequence
  Nucleotide sequence of the transaminase ATA117_ACHH
atggcatttagcgcggataccagcgaaatcgtctatacccacgataccggtctggattacatcacctacagcgattacgaactggatccggcaaatccgttagcaggcggcgcagcttggattgaaggcgcatttgttccgccgtctgaagcgcgtattagcatcttcgatcagggctatctgcatagcgacgttacctataccgcattccacgtttggaacggtaacgcatttcgtctggacgatcacatcgaacgtctgttcagcaacgccgaaagtatgcgtattattccgccgctgacccaagacgaagtcaaagaaatcgcgctggaactggttgcaaaaaccgaactgcgcgaagcgtgtgttagcgttagcattacccgcggttatagtagtaccccgggcgaacgcgatattaccaaacatcgtccgcaggtctacatgtacgctgttccgtaccagtggcatgttccgtttgatcgtattcgcgacggcgttcacgcaatggttgcacagagcgtgcgtcgtaccccgcgtagcagcatcgatccgcaggtcaaaaacttccagtggggcgatttaattcgcgcagttcaggaaacccacgatcgcggttttgaagcaccgttactgttagacggcgacggtttactggcagaaggtagcggccataacgtcgtcgtcattaaagatggggttgttcgttctccgggtcgtgcagcattaccgggtattacccgcaaaaccgttctggaaattgcggaatccctgggtcatgaagcgattctggcggatattaccttagcggaactgctggacgcagacgaagttttaggttgtaccaccgctggcggcgtttggccgtttgttagcgttgacggcaatccgattagcgatggtgttccgggtccggttacccaaagcattattcgtcgctactgggagctgaacgttgaaagtagcagcctgttaaccccggttcagtattaa

SEQ ID NO: 7 - protein, 663 aa, Artificial Sequence
  Amino acid sequence of the transketolase EcTK1_YYH
MSSRKELANAIRALSMDAVQKAKSGYPGAPMGMADIAEVLWRDFLKHNPQNPSWADRDRFVLSNGHGSMLIYSLLHLTGYDLPMEELKNFRQLHSKTPGHPEVGYTAGVETTTGPLGQGIANAVGMAIAEKTLAAQFNRPGHDIVDHYTYAFMGDGCMMEGISHEVCSLAGTLKLGKLIAFYDDNGISIDGHVEGWFTDDTAMRFEAYGWHVIRDIDGHDAASIKRAVEEARAVTDKPSLLMCKTIIGFGSPNKAGTHDSHGAPLGDAEIALTREQLGWKYAPFEIPSEIYAQWDAKEAGQAKESAWNEKFAAYAKAYPQEAAEFTRRMKGEMPSDFDAKAKEFIAKLQANPAKIASRKASQNAIEAFGPLLPEFLGGSADLAPYNLTLWSGSKAINEDAAGNYIHYGVREFGMTAIANGISLHGGFLPYTSTYLMFVEYARNAVRMAALMKQRQVMVYTHDSIGHGETGPTHQPVEQVASLRVTPNMSTWRPCDQVESAVAWKYGVERQDGPTALILSQQNLAQQERTEEQLANIARGGYVLKDCAGQPELIFIATGSEVELAVAAYEKLTAEGVKARVVSMPSTDAFDKQDAAYRESVLPKAVTARVAVEAGIADYWYKYVGLNGAIVGMTTFGESAPAELLFEEFGFTVDNVVAKAKELL

SEQ ID NO: 8 - protein, 330 aa, Artificial Sequence
  Amino acid sequence of the transaminase ATA117_ACHH
MAFSADTSEIVYTHDTGLDYITYSDYELDPANPLAGGAAWIEGAFVPPSEARISIFDQGYLHSDVTYTAFHVWNGNAFRLDDHIERLFSNAESMRIIPPLTQDEVKEIALELVAKTELREACVSVSITRGYSSTPGERDITKHRPQVYMYAVPYQWHVPFDRIRDGVHAMVAQSVRRTPRSSIDPQVKNFQWGDLIRAVQETHDRGFEAPLLLDGDGLLAEGSGHNVVVIKDGVVRSPGRAALPGITRKTVLEIAESLGHEAILADITLAELLDADEVLGCTTAGGVWPFVSVDGNPISDGVPGPVTQSIIRRYWELNVESSSLLTPVQY